European Patent Application EP 4 603 512 A1, published August 20, 2025. Title: B7H3/PDL1 BISPECIFIC ANTIBODY, AND PHARMACEUTICAL COMPOSITION COMPRISING SAME AND USE THEREOF. Applicant: DARTSBIO PHARMACEUTICALS LTD. Application WO PCT/CN2022/125089, filed October 13, 2022. The sequence listing filed with the application follows.

SEQUENCE LISTING (17 sequences)

SEQ ID NO: 1 - protein, 11 aa, synthetic construct
RASQSINTYLH

SEQ ID NO: 2 - protein, 7 aa, synthetic construct
YASQSIS

SEQ ID NO: 3 - protein, 9 aa, synthetic construct
QNGHSFPLT

SEQ ID NO: 4 - protein, 107 aa, synthetic construct
DIQMTQSPSSLSASVGDRVTISCRASQSINTYLHWYQQKLGQAPRLLIYYASQSISGVPSRFSGSGSGTDFTLTINSLEAEDAATYYCQNGHSFPLTFGAGTKVEIK

SEQ ID NO: 5 - protein, 5 aa, synthetic construct
TFGVH

SEQ ID NO: 6 - protein, 16 aa, synthetic construct
IIWPGGNTNYNSALMS

SEQ ID NO: 7 - protein, 9 aa, synthetic construct
ENYGRAMDY

SEQ ID NO: 8 - protein, 117 aa, synthetic construct
QVQLVQSGAEVKKPGASVKVSCKASGYTFTTFGVHWVRQAPGKGLEWVGIIWPGGNTNYNSALMSRVTITADESTSTAYMELSSLRSEDTAVYYCARENYGRAMDYWGQGTTVTVSS

SEQ ID NO: 9 - protein, 214 aa, synthetic construct
DIQMTQSPSSLSASVGDRVTISCRASQSINTYLHWYQQKLGQAPRLLIYYASQSISGVPSRFSGSGSGTDFTLTINSLEAEDAATYYCQNGHSFPLTFGAGTKVEIKRTVAAPSVFIFPPSDEQLKSGTASVVCLLNNFYPREAKVQWKVDNALQSGNSQESVTEQDSKDSTYSLSSTLTLSKADYEKHKVYACEVTHQGLSSPVTKSFNRGEC

SEQ ID NO: 10 - protein, 447 aa, synthetic construct
QVQLVQSGAEVKKPGASVKVSCKASGYTFTTFGVHWVRQAPGKGLEWVGIIWPGGNTNYNSALMSRVTITADESTSTAYMELSSLRSEDTAVYYCARENYGRAMDYWGQGTTVTVSSASTKGPSVFPLAPSSKSTSGGTAALGCLVKDYFPEPVTVSWNSGALTSGVHTFPAVLQSSGLYSLSSVVTVPSSSLGTQTYICNVNHKPSNTKVDKKVEPKSCDKTHTCPPCPAPELLGGPSVFLFPPKPKDTLMISRTPEVTCVVVDVSHEDPEVKFNWYVDGVEVHNAKTKPREEQYNSTYRVVSVLTVLHQDWLNGKEYKCKVSNKALPAPIEKTISKAKGQPREPQVYTLPPSREEMTKNQVSLTCLVKGFYPSDIAVEWESNGQPENNYKTTPPVLDSDGSFFLYSKLTVDKSRWQQGNVFSCSVMHEALHNHYTQKSLSLSPGK

SEQ ID NO: 11 - protein, 15 aa, synthetic construct
GGGGSGGGGTGGGGS

SEQ ID NO: 12 - protein, 5 aa, synthetic construct
TIWIG

SEQ ID NO: 13 - protein, 17 aa, unidentified
AIYIGSGATYYVDSVKG

SEQ ID NO: 14 - protein, 19 aa, synthetic construct
TGGTVGSMVRFSPVGDFGY

SEQ ID NO: 15 - protein, 128 aa, synthetic construct
DVQLQESGGGLVQAGGSLRLSCTASGYTLSTIWIGWFRQAPGKGLEGVAAIYIGSGATYYVDSVKGRFTISQDNAKNTVYLQMNSLKPEDTAMYYCAATGGTVGSMVRFSPVGDFGYWGQGTQVTVSS

SEQ ID NO: 16 - protein, 590 aa, synthetic construct
QVQLVQSGAEVKKPGASVKVSCKASGYTFTTFGVHWVRQAPGKGLEWVGIIWPGGNTNYNSALMSRVTITADESTSTAYMELSSLRSEDTAVYYCARENYGRAMDYWGQGTTVTVSSASTKGPSVFPLAPSSKSTSGGTAALGCLVKDYFPEPVTVSWNSGALTSGVHTFPAVLQSSGLYSLSSVVTVPSSSLGTQTYICNVNHKPSNTKVDKKVEPKSCDKTHTCPPCPAPELLGGPSVFLFPPKPKDTLMISRTPEVTCVVVDVSHEDPEVKFNWYVDGVEVHNAKTKPREEQYNSTYRVVSVLTVLHQDWLNGKEYKCKVSNKALPAPIEKTISKAKGQPREPQVYTLPPSREEMTKNQVSLTCLVKGFYPSDIAVEWESNGQPENNYKTTPPVLDSDGSFFLYSKLTVDKSRWQQGNVFSCSVMHEALHNHYTQKSLSLSPGKGGGGSGGGGTGGGGSDVQLQESGGGLVQAGGSLRLSCTASGYTLSTIWIGWFRQAPGKGLEGVAAIYIGSGATYYVDSVKGRFTISQDNAKNTVYLQMNSLKPEDTAMYYCAATGGTVGSMVRFSPVGDFGYWGQGTQVTVSS

SEQ ID NO: 17 - protein, 214 aa, synthetic construct; identical to SEQ ID NO: 9